European Patent Application EP 4 170 042 A1, published April 26, 2023. Title: METHODS FOR THE DIAGNOSIS OF FETAL ABNORMALITIES. Applicant: Verinata Health, Inc. Application EP TBC, filed September 6, 2022. The sequence listing filed with the application follows.

SEQUENCE LISTING (172 sequences)

SEQ ID NO: 1 - DNA, 20 bp, synthetic construct
  source 1..20: mol_type = other DNA
acagaagtctgggatgtgga

SEQ ID NO: 2 - DNA, 20 bp, synthetic construct
  source 1..20: mol_type = other DNA
gcccaaaaagacagacagaa

SEQ ID NO: 3 - DNA, 20 bp, synthetic construct
  source 1..20: mol_type = other DNA
acctgttgtatggcagcagt

SEQ ID NO: 4 - DNA, 21 bp, synthetic construct
  source 1..21: mol_type = other DNA
agttgactctttccccaacta

SEQ ID NO: 5 - DNA, 22 bp, synthetic construct
  source 1..22: mol_type = other DNA
tttggtaagaaaaacatctccc

SEQ ID NO: 6 - DNA, 20 bp, synthetic construct
  source 1..20: mol_type = other DNA
ggctgcagttagctgtcatt

SEQ ID NO: 7 - DNA, 19 bp, synthetic construct
  source 1..19: mol_type = other DNA
cctgggcaacaagagcaaa

SEQ ID NO: 8 - DNA, 20 bp, synthetic construct
  source 1..20: mol_type = other DNA
agcagagagacataattgtg

SEQ ID NO: 9 - DNA, 20 bp, synthetic construct
  source 1..20: mol_type = other DNA
acctgccaaattttaccagg

SEQ ID NO: 10 - DNA, 21 bp, synthetic construct
  source 1..21: mol_type = other DNA
gacagagagagggaataaacc

SEQ ID NO: 11 - DNA, 21 bp, synthetic construct
  source 1..21: mol_type = other DNA
atatatgcacatccatccatg

SEQ ID NO: 12 - DNA, 23 bp, synthetic construct
  source 1..23: mol_type = other DNA
ggccaaagatagatagcaaggta

SEQ ID NO: 13 - DNA, 20 bp, synthetic construct
  source 1..20: mol_type = other DNA
acatcgctccttaccccatc

SEQ ID NO: 14 - DNA, 21 bp, synthetic construct
  source 1..21: mol_type = other DNA
tgtacccattaaccatcccca

SEQ ID NO: 15 - DNA, 20 bp, synthetic construct
  source 1..20: mol_type = other DNA
acagaagtctgggatgtgga

SEQ ID NO: 16 - DNA, 20 bp, synthetic construct
  source 1..20: mol_type = other DNA
gcccaaaaagacagacagaa

SEQ ID NO: 17 - DNA, 24 bp, synthetic construct
  source 1..24: mol_type = other DNA
agagtgagattctgtctcaattaa

SEQ ID NO: 18 - DNA, 20 bp, synthetic construct
  source 1..20: mol_type = other DNA
ggccctgtgtagaagctgta

SEQ ID NO: 19 - DNA, 20 bp, synthetic construct
  source 1..20: mol_type = other DNA
atcaggattccaggaggaaa

SEQ ID NO: 20 - DNA, 18 bp, synthetic construct
  source 1..18: mol_type = other DNA
acctgggaggcggagctc

SEQ ID NO: 21 - DNA, 23 bp, synthetic construct
  source 1..23: mol_type = other DNA
ggcataaaaatagtacagcaagc

SEQ ID NO: 22 - DNA, 20 bp, synthetic construct
  source 1..20: mol_type = other DNA
atttgaacagaggcatgtac

SEQ ID NO: 23 - DNA, 20 bp, synthetic construct
  source 1..20: mol_type = other DNA
catggatgcagaattcacag

SEQ ID NO: 24 - DNA, 20 bp, synthetic construct
  source 1..20: mol_type = other DNA
tcatctccctgtttggtagc

SEQ ID NO: 25 - DNA, 21 bp, synthetic construct
  source 1..21: mol_type = other DNA
agggatcttcagagaaacagg

SEQ ID NO: 26 - DNA, 21 bp, synthetic construct
  source 1..21: mol_type = other DNA
tgacactatcagctctctggc

SEQ ID NO: 27 - DNA, 23 bp, synthetic construct
  source 1..23: mol_type = other DNA
ggtgcttgctgtaaatataattg

SEQ ID NO: 28 - DNA, 20 bp, synthetic construct
  source 1..20: mol_type = other DNA
cactacagcagattgcacca

SEQ ID NO: 29 - DNA, 20 bp, synthetic construct
  source 1..20: mol_type = other DNA
caaacccgactaccagcaac

SEQ ID NO: 30 - DNA, 20 bp, synthetic construct
  source 1..20: mol_type = other DNA
gagccatgttcatgccactg

SEQ ID NO: 31 - DNA, 26 bp, synthetic construct
  source 1..26: mol_type = other DNA
caaagagtgaatgctgtacaaacagc

SEQ ID NO: 32 - DNA, 26 bp, synthetic construct
  source 1..26: mol_type = other DNA
caagatgtgagtgtgcttttcaggag

SEQ ID NO: 33 - DNA, 20 bp, synthetic construct
  source 1..20: mol_type = other DNA
atcccacaggatgcctattt

SEQ ID NO: 34 - DNA, 20 bp, synthetic construct
  source 1..20: mol_type = other DNA
acgggagcttttgagaagtt

SEQ ID NO: 35 - DNA, 23 bp, synthetic construct
  source 1..23: mol_type = other DNA
tcaaatttttaagtctcaccagg

SEQ ID NO: 36 - DNA, 20 bp, synthetic construct
  source 1..20: mol_type = other DNA
gcctgtagaaagcaacaacc

SEQ ID NO: 37 - DNA, 20 bp, synthetic construct
  source 1..20: mol_type = other DNA
ggtgacagagcaagaccttg

SEQ ID NO: 38 - DNA, 20 bp, synthetic construct
  source 1..20: mol_type = other DNA
gcctcttgtcatcccaagta

SEQ ID NO: 39 - DNA, 20 bp, synthetic construct
  source 1..20: mol_type = other DNA
ctctcttcatccaccattgg

SEQ ID NO: 40 - DNA, 20 bp, synthetic construct
  source 1..20: mol_type = other DNA
gctgtaagagacctgtgttg

SEQ ID NO: 41 - DNA, 20 bp, synthetic construct
  source 1..20: mol_type = other DNA
tggaaccacttcattcttgg

SEQ ID NO: 42 - DNA, 19 bp, synthetic construct
  source 1..19: mol_type = other DNA
atttcagaccaagataggc

SEQ ID NO: 43 - DNA, 21 bp, synthetic construct
  source 1..21: mol_type = other DNA
cctatttaagtttctgtaagg

SEQ ID NO: 44 - DNA, 20 bp, synthetic construct
  source 1..20: mol_type = other DNA
atggtgtagaccctgtggaa

SEQ ID NO: 45 - DNA, 22 bp, synthetic construct
  source 1..22: mol_type = other DNA
ctgcacaacatagtgagacctg

SEQ ID NO: 46 - DNA, 24 bp, synthetic construct
  source 1..24: mol_type = other DNA
agattacccagaaatgagatcagc

SEQ ID NO: 47 - DNA, 20 bp, synthetic construct
  source 1..20: mol_type = other DNA
tcatgtgacaaaagccacac

SEQ ID NO: 48 - DNA, 25 bp, synthetic construct
  source 1..25: mol_type = other DNA
agacagaaatatagatgagaatgca

SEQ ID NO: 49 - DNA, 20 bp, synthetic construct
  source 1..20: mol_type = other DNA
tcatgtgacaaaagccacac

SEQ ID NO: 50 - DNA, 25 bp, synthetic construct
  source 1..25: mol_type = other DNA
agacagaaatatagatgagaatgca

SEQ ID NO: 51 - DNA, 20 bp, synthetic construct
  source 1..20: mol_type = other DNA
tttccagtggaaaccaaact

SEQ ID NO: 52 - DNA, 20 bp, synthetic construct
  source 1..20: mol_type = other DNA
tccagcaacaacaagagaca

SEQ ID NO: 53 - DNA, 21 bp, synthetic construct
  source 1..21: mol_type = other DNA
gtcctcatcctgtaaaacggg

SEQ ID NO: 54 - DNA, 24 bp, synthetic construct
  source 1..24: mol_type = other DNA
ccactaactagtttgtgactttgg

SEQ ID NO: 55 - DNA, 22 bp, synthetic construct
  source 1..22: mol_type = other DNA
ctgtcctctaggctcatttagc

SEQ ID NO: 56 - DNA, 20 bp, synthetic construct
  source 1..20: mol_type = other DNA
ttatgaagcagtgatgccaa

SEQ ID NO: 57 - DNA, 20 bp, synthetic construct
  source 1..20: mol_type = other DNA
agctggagagggatagcatt

SEQ ID NO: 58 - DNA, 20 bp, synthetic construct
  source 1..20: mol_type = other DNA
tgcattgcatgaaagtagga

SEQ ID NO: 59 - DNA, 21 bp, synthetic construct
  source 1..21: mol_type = other DNA
gatgatagagatggcacatga

SEQ ID NO: 60 - DNA, 23 bp, synthetic construct
  source 1..23: mol_type = other DNA
tcttcatacatgctttatcatgc

SEQ ID NO: 61 - DNA, 18 bp, synthetic construct
  source 1..18: mol_type = other DNA
gtgagtcaattccccaag

SEQ ID NO: 62 - DNA, 22 bp, synthetic construct
  source 1..22: mol_type = other DNA
gttgtattagtcaatgttctcc

SEQ ID NO: 63 - DNA, 22 bp, synthetic construct
  source 1..22: mol_type = other DNA
atgatgaatgcatagatggatg

SEQ ID NO: 64 - DNA, 19 bp, synthetic construct
  source 1..19: mol_type = other DNA
aatgtgtgtccttccaggc

SEQ ID NO: 65 - DNA, 19 bp, synthetic construct
  source 1..19: mol_type = other DNA
ttgcagggaaaccacagtt

SEQ ID NO: 66 - DNA, 20 bp, synthetic construct
  source 1..20: mol_type = other DNA
tccttggaataaattcccgg

SEQ ID NO: 67 - DNA, 24 bp, synthetic construct
  source 1..24: mol_type = other DNA
cttagagggacagaactaataggc

SEQ ID NO: 68 - DNA, 20 bp, synthetic construct
  source 1..20: mol_type = other DNA
agcctattgtgggtttgtga

SEQ ID NO: 69 - DNA, 21 bp, synthetic construct
  source 1..21: mol_type = other DNA
atgtacatgtgtctgggaagg

SEQ ID NO: 70 - DNA, 24 bp, synthetic construct
  source 1..24: mol_type = other DNA
ttctctacatatttactgccaaca

SEQ ID NO: 71 - DNA, 24 bp, synthetic construct
  source 1..24: mol_type = other DNA
gagtttgaaaataaagtgttctgc

SEQ ID NO: 72 - DNA, 20 bp, synthetic construct
  source 1..20: mol_type = other DNA
ccccaccccttttagtttta

SEQ ID NO: 73 - DNA, 25 bp, synthetic construct
  source 1..25: mol_type = other DNA
atgtacgatacgtaatacttgacaa

SEQ ID NO: 74 - DNA, 18 bp, synthetic construct
  source 1..18: mol_type = other DNA
gtcccaaaggacctgctc

SEQ ID NO: 75 - DNA, 21 bp, synthetic construct
  source 1..21: mol_type = other DNA
gcacccctttatacttgggtg

SEQ ID NO: 76 - DNA, 25 bp, synthetic construct
  source 1..25: mol_type = other DNA
tagtactctaccatccatctatccc

SEQ ID NO: 77 - DNA, 24 bp, synthetic construct
  source 1..24: mol_type = other DNA
aacagaaccaataggctatctatc

SEQ ID NO: 78 - DNA, 24 bp, synthetic construct
  source 1..24: mol_type = other DNA
tacagtaaatcacttggtaggaga

SEQ ID NO: 79 - DNA, 17 bp, synthetic construct
  source 1..17: mol_type = other DNA
tccgcgaagtgaagaac

SEQ ID NO: 80 - DNA, 20 bp, synthetic construct
  source 1..20: mol_type = other DNA
cttggggagaaccatcctca

SEQ ID NO: 81 - DNA, 20 bp, synthetic construct
  source 1..20: mol_type = other DNA
ccggctacaagtgatgtcta

SEQ ID NO: 82 - DNA, 24 bp, synthetic construct
  source 1..24: mol_type = other DNA
cctaggtaacatagtgagaccttg

SEQ ID NO: 83 - DNA, 20 bp, synthetic construct
  source 1..20: mol_type = other DNA
cctctaaagcatagggtcca

SEQ ID NO: 84 - DNA, 19 bp, synthetic construct
  source 1..19: mol_type = other DNA
cccatctgagaacacgctg

SEQ ID NO: 85 - DNA, 23 bp, synthetic construct
  source 1..23: mol_type = other DNA
agtttaggagattatcaagctgg

SEQ ID NO: 86 - DNA, 23 bp, synthetic construct
  source 1..23: mol_type = other DNA
gttcccataatagatgtatccag

SEQ ID NO: 87 - DNA, 24 bp, synthetic construct
  source 1..24: mol_type = other DNA
ttggtacttaataaaccctctttt

SEQ ID NO: 88 - DNA, 22 bp, synthetic construct
  source 1..22: mol_type = other DNA
ctagagggacagaaccaatagg

SEQ ID NO: 89 - DNA, 22 bp, synthetic construct
  source 1..22: mol_type = other DNA
tgtctgctaatgaatgatttgg

SEQ ID NO: 90 - DNA, 20 bp, synthetic construct
  source 1..20: mol_type = other DNA
ccatcccctaaacctctcat

SEQ ID NO: 91 - DNA, 20 bp, synthetic construct
  source 1..20: mol_type = other DNA
gtgggaccttgtgattgtgt

SEQ ID NO: 92 - DNA, 20 bp, synthetic construct
  source 1..20: mol_type = other DNA
ctggctgacacttagggaaa

SEQ ID NO: 93 - DNA, 20 bp, synthetic construct
  source 1..20: mol_type = other DNA
acagaaaaccttttgggacc

SEQ ID NO: 94 - DNA, 20 bp, synthetic construct
  source 1..20: mol_type = other DNA
cccagccctgaatattatca

SEQ ID NO: 95 - DNA, 22 bp, synthetic construct
  source 1..22: mol_type = other DNA
tgcacttaatatctggtgatgg

SEQ ID NO: 96 - DNA, 20 bp, synthetic construct
  source 1..20: mol_type = other DNA
atttctttccctctgcaacc

SEQ ID NO: 97 - DNA, 22 bp, synthetic construct
  source 1..22: mol_type = other DNA
agcccattttcataataaatcc

SEQ ID NO: 98 - DNA, 24 bp, synthetic construct
  source 1..24: mol_type = other DNA
aatcagtgctttctgtactattgg

SEQ ID NO: 99 - DNA, 20 bp, synthetic construct
  source 1..20: mol_type = other DNA
cacttcatggcttaccacag

SEQ ID NO: 100 - DNA, 20 bp, synthetic construct
  source 1..20: mol_type = other DNA
gacctttggaaagctagtgt

SEQ ID NO: 101 - DNA, 20 bp, synthetic construct
  source 1..20: mol_type = other DNA
tgtcacgtttaccctggaac

SEQ ID NO: 102 - DNA, 23 bp, synthetic construct
  source 1..23: mol_type = other DNA
tattcttctatccaaccaacagc

SEQ ID NO: 103 - DNA, 18 bp, synthetic construct
  source 1..18: mol_type = other DNA
ttgggtggggacacagag

SEQ ID NO: 104 - DNA, 20 bp, synthetic construct
  source 1..20: mol_type = other DNA
cctggctcaaggaattacaa

SEQ ID NO: 105 - DNA, 20 bp, synthetic construct
  source 1..20: mol_type = other DNA
ccagcctggctgttagagta

SEQ ID NO: 106 - DNA, 25 bp, synthetic construct
  source 1..25: mol_type = other DNA
atattcttatattccatatggcaca

SEQ ID NO: 107 - DNA, 20 bp, synthetic construct
  source 1..20: mol_type = other DNA
tggagtctctgggtgaagag

SEQ ID NO: 108 - DNA, 20 bp, synthetic construct
  source 1..20: mol_type = other DNA
caggagtatgggatcaccag

SEQ ID NO: 109 - DNA, 18 bp, synthetic construct
  source 1..18: mol_type = other DNA
cagcaatttttcaaaggc

SEQ ID NO: 110 - DNA, 25 bp, synthetic construct
  source 1..25: mol_type = other DNA
agatcattcatataacctcaaaaga

SEQ ID NO: 111 - DNA, 17 bp, synthetic construct
  source 1..17: mol_type = other DNA
ttgctgctggtggtggc

SEQ ID NO: 112 - DNA, 20 bp, synthetic construct
  source 1..20: mol_type = other DNA
cagggattccgtcatatggc

SEQ ID NO: 113 - DNA, 18 bp, synthetic construct
  source 1..18: mol_type = other DNA
gatcggcctcttcatgcg

SEQ ID NO: 114 - DNA, 22 bp, synthetic construct
  source 1..22: mol_type = other DNA
gatccaaaggtcatcaactccc

SEQ ID NO: 115 - DNA, 18 bp, synthetic construct
  source 1..18: mol_type = other DNA
gctgtccaacgaatgggc

SEQ ID NO: 116 - DNA, 20 bp, synthetic construct
  source 1..20: mol_type = other DNA
ggcgttctcctttctccagg

SEQ ID NO: 117 - DNA, 19 bp, synthetic construct
  source 1..19: mol_type = other DNA
atgcactgggccaggtctt

SEQ ID NO: 118 - DNA, 21 bp, synthetic construct
  source 1..21: mol_type = other DNA
cgatggtacatatgggtggct

SEQ ID NO: 119 - DNA, 19 bp, synthetic construct
  source 1..19: mol_type = other DNA
aggctgtccaacgaatggg

SEQ ID NO: 120 - DNA, 19 bp, synthetic construct
  source 1..19: mol_type = other DNA
ctgagggaggcgttctcct

SEQ ID NO: 121 - DNA, 22 bp, synthetic construct
  source 1..22: mol_type = other DNA
tcagagcctgtgtttctaccaa

SEQ ID NO: 122 - DNA, 22 bp, synthetic construct
  source 1..22: mol_type = other DNA
tggtctcacaggaccactgatt

SEQ ID NO: 123 - DNA, 20 bp, synthetic construct
  source 1..20: mol_type = other DNA
tccaaatgagctggcaagtg

SEQ ID NO: 124 - DNA, 23 bp, synthetic construct
  source 1..23: mol_type = other DNA
tcccaaacactcagtgaaacaaa

SEQ ID NO: 125 - DNA, 24 bp, synthetic construct
  source 1..24: mol_type = other DNA
aaataatcagtgtgattcgtggag

SEQ ID NO: 126 - DNA, 22 bp, synthetic construct
  source 1..22: mol_type = other DNA
gaggccagtgctgtctctaagg

SEQ ID NO: 127 - DNA, 20 bp, synthetic construct
  source 1..20: mol_type = other DNA
gtgcatcgctggtaacatcc

SEQ ID NO: 128 - DNA, 20 bp, synthetic construct
  source 1..20: mol_type = other DNA
tgtggagatgagcagggtct

SEQ ID NO: 129 - DNA, 21 bp, synthetic construct
  source 1..21: mol_type = other DNA
acttcacagccctgcgtaaac

SEQ ID NO: 130 - DNA, 21 bp, synthetic construct
  source 1..21: mol_type = other DNA
atgggacaggcactgatttgt

SEQ ID NO: 131 - DNA, 20 bp, synthetic construct
  source 1..20: mol_type = other DNA
atcgcattcatgcgtcttca

SEQ ID NO: 132 - DNA, 20 bp, synthetic construct
  source 1..20: mol_type = other DNA
atccccatggcaaactcttg

SEQ ID NO: 133 - DNA, 22 bp, synthetic construct
  source 1..22: mol_type = other DNA
gcagcgggttacatcttctttc

SEQ ID NO: 134 - DNA, 22 bp, synthetic construct
  source 1..22: mol_type = other DNA
cagctctggctcacactaccag

SEQ ID NO: 135 - DNA, 22 bp, synthetic construct
  source 1..22: mol_type = other DNA
gcagcgggttacatcttctttc

SEQ ID NO: 136 - DNA, 19 bp, synthetic construct
  source 1..19: mol_type = other DNA
catcctcccctgcatgtgt

SEQ ID NO: 137 - DNA, 20 bp, synthetic construct
  source 1..20: mol_type = other DNA
ccgcagcatgtcaagatcac

SEQ ID NO: 138 - DNA, 25 bp, synthetic construct
  source 1..25: mol_type = other DNA
tccttctgcatggtattctttctct

SEQ ID NO: 139 - DNA, 14 bp, synthetic construct
  source 1..14: mol_type = other DNA
tttgggctggccaa

SEQ ID NO: 140 - DNA, 14 bp, synthetic construct
  source 1..14: mol_type = other DNA
ttttgggcgggcca

SEQ ID NO: 141 - DNA, 17 bp, synthetic construct
  source 1..17: mol_type = other DNA
atggccagcgtggacaa

SEQ ID NO: 142 - DNA, 23 bp, synthetic construct
  source 1..23: mol_type = other DNA
agcaggtactgggagccaatatt

SEQ ID NO: 143 - DNA, 16 bp, synthetic construct
  source 1..16: mol_type = other DNA
atgagctgcgtgatga

SEQ ID NO: 144 - DNA, 16 bp, synthetic construct
  source 1..16: mol_type = other DNA
atgagctgcatgatga

SEQ ID NO: 145 - DNA, 22 bp, synthetic construct
  source 1..22: mol_type = other DNA
gcctcttacacccagtggagaa

SEQ ID NO: 146 - DNA, 22 bp, synthetic construct
  source 1..22: mol_type = other DNA
ttctgggatccagagtccctta

SEQ ID NO: 147 - DNA, 14 bp, synthetic construct
  source 1..14: mol_type = other DNA
accggagcccagca

SEQ ID NO: 148 - DNA, 14 bp, synthetic construct
  source 1..14: mol_type = other DNA
accggagctcagca

SEQ ID NO: 149 - DNA, 14 bp, synthetic construct
  source 1..14: mol_type = other DNA
accggagcacagca

SEQ ID NO: 150 - DNA, 21 bp, synthetic construct
  source 1..21: mol_type = other DNA
tcgcaaagggcatgaactact

SEQ ID NO: 151 - DNA, 21 bp, synthetic construct
  source 1..21: mol_type = other DNA
atcttgacatgctgcggtgtt

SEQ ID NO: 152 - DNA, 14 bp, synthetic construct
  source 1..14: mol_type = other DNA
ttggtgcaccgcga

SEQ ID NO: 153 - DNA, 14 bp, synthetic construct
  source 1..14: mol_type = other DNA
tggtgctccgcgac

SEQ ID NO: 154 - DNA, 19 bp, synthetic construct
  source 1..19: mol_type = other DNA
agtcaggacccatgcacgg

SEQ ID NO: 155 - DNA, 20 bp, synthetic construct
  source 1..20: mol_type = other DNA
acccaagatgcagcagtgtg

SEQ ID NO: 156 - DNA, 21 bp, synthetic construct
  source 1..21: mol_type = other DNA
gatgtcctccttgttctactc

SEQ ID NO: 157 - DNA, 22 bp, synthetic construct
  source 1..22: mol_type = other DNA
tacagggaataatcgagcatgc

SEQ ID NO: 158 - DNA, 22 bp, synthetic construct
  source 1..22: mol_type = other DNA
gaagggaaatagcaaatggaca

SEQ ID NO: 159 - DNA, 20 bp, synthetic construct
  source 1..20: mol_type = other DNA
cgatggagtccaagttctgg

SEQ ID NO: 160 - DNA, 20 bp, synthetic construct
  source 1..20: mol_type = other DNA
agcacttacagctctggcca

SEQ ID NO: 161 - DNA, 22 bp, synthetic construct
  source 1..22: mol_type = other DNA
gactgaacataactgtaggctg

SEQ ID NO: 162 - DNA, 19 bp, synthetic construct
  source 1..19: mol_type = other DNA
tcgagtgcattccattccg

SEQ ID NO: 163 - DNA, 21 bp, synthetic construct
  source 1..21: mol_type = other DNA
atggaatggcatcaaacggaa

SEQ ID NO: 164 - DNA, 15 bp, synthetic construct
  source 1..15: mol_type = other DNA
tggctgtccattcca

SEQ ID NO: 165 - DNA, 65 bp, synthetic construct
  source 1..65: mol_type = other DNA
atgcagcaaggcacagactaarcaaggagasgcaaaattttcrtaggggagagaaatgggtcatt

SEQ ID NO: 166 - DNA, 22 bp, synthetic construct
  source 1..22: mol_type = other DNA
atgcagcaaggcacagactacg

SEQ ID NO: 167 - DNA, 23 bp, synthetic construct
  source 1..23: mol_type = other DNA
agaggggagagaaatgggtcatt

SEQ ID NO: 168 - DNA, 25 bp, synthetic construct
  source 1..25: mol_type = other DNA
caaggcacagactaagcaaggagag

SEQ ID NO: 169 - DNA, 35 bp, synthetic construct
  source 1..35: mol_type = other DNA
ggcaaaattttcataggggagagaaatgggtcatt

SEQ ID NO: 170 - DNA, 15 bp, synthetic construct
  source 1..15: mol_type = other DNA
gcaactcatcatgca

SEQ ID NO: 171 - DNA, 15 bp, synthetic construct
  source 1..15: mol_type = other DNA
ttttgggcgggccaa

SEQ ID NO: 172 - DNA, 19 bp, synthetic construct
  source 1..19: mol_type = other DNA
gaccgtttgggagttgata